European Patent Application EP 4 534 673 A1, published April 9, 2025. Title: NUCLEIC ACID MODIFIED TO OBTAIN ENHANCED ERGOTHIONEINE PRODUCTIVITY, AND MICROORGANISM HAVING GENETIC MODIFICATION. Applicant: Kikkoman Corporation. Application EP 23816064.2, filed May 30, 2023. The sequence listing filed with the application follows.

SEQUENCE LISTING (79 sequences)

SEQ ID NO: 1 - protein, 657 aa, Aspergillus oryzae
MTSSASHHQHSSTSAAEFSTHQTAPSSNIDPNGNIATSGYAPNESQLAGLVEAATAAAGQDVSEWAAAAAVAAAAGAAGHQHHLDGYPPDIHIEDDSFADAGFGTGLSTGRQLRAPGPSPNEHSQPSGLSRTVSKKRKRDGPLDPALTASGPGGHQQPHQHNSHHYGGETLDIRSAPPQSLSEARAVGLHSAAALFRQPSSNKKYTRPPMSKLFASLELSPENFLHLQAAAKSYMLDDKHPERRECVGQRGKGDTEMVKLRLWNCVRHFLEIEGHGERFFGENVVNEGMGPRTYVWPRDQQKIIALVIPLLRRMVTNERQRQYAVETRKGGGSEERRRRKTEDSLQNMNSASPPKFPVEEQLQMHAQHHPPEGYAPTHPELGATSQDMELGLTDLLPDGYPADWNAISKTYEAYNQNYELDNLWYLSGLQQPDWRGLVAAVDSHYQVFHNGSFDCPAPCEDENINHILHANSVSGLRWRVGGDRHQVARNEFASSITRDVSRIIRDNIATKHGVQTSTDDHAPIHPSNFPPLPTGLTMPNPPTTSQAPISLRINIMQNGKRVLPRVDLPAGHCPDLETLKQLLCRRFAGQLPGLPSDPSLDPAAWMSSVGWRFRVWLPEGLTPVQNDGEWTIALLSAGNVDWMDGDLRVLVELENTS

SEQ ID NO: 2 - DNA, 2038 bp, Aspergillus oryzae
  source 1..2038: mol_type = genomic DNA
atgacgtcttctgcttcccatcaccaacattcttcgacttcagccgctgaattttccactcaccaaaccgctccttcctccaacatcgacccgaacggtaacattgccacgagtggatatgcgccaaatgaaagccaacttgctgggctggtagaagctgctactgcagcggctggccaggatgtatcggaatgggcggccgccgctgcagtcgctgctgcagctggtgctgccggacatcagcatcatttagacggctaccccccggatattcatatcgaagacgatagttttgcagatgcaggttttgggacagggttgagcactggaagacagttacgagcacccgggccatctcccaacgagcatagccagccttcgggactgtcaagaactgtgtcaaagaagagaaagagagatggccctctagacccagccttaacagcgtctggacctggtggtcaccagcagccccatcagcacaattctcatcattatggtggtgagacgctagatatccggtctgcacctccccagtccttatcggaggcgcgcgctgttggtttacattccgcagctgctttgttccgtcaaccctcgagcaacaagaagtacacacgaccacctatgtcgaagctttttgcttcactcgaactatcaccggagaacttcctccacttacaagccgctgctaagtcatatatgctagatgacaagcatccagaacgacgtgagtgtgtcggtcaacgtggcaagggagacacggaaatggttaaactgagactttggaattgtgtgcgccactttctcgaaattgaggggcatggtgaacgttttttcggtgaaaatgtagtcaacgagggcatgggtcccaggacctatgtatggccccgggaccagcaaaaaattattgcacttgtcattccactgctacggcgtatggtcaccaatgaacgacagagacaatatgcagtggagacgaggaaggggggtggatctgaggagcgacgacgacggaaaaccgaagacagtctccagaatatgaatagtgctagtcctccgaagttccccgttgaggaacaactccagatgcatgcgcaacatcatcctcccgaggggtatgcgccaacacaccccgagttgggggcaacttcccaagacatggagttgggcctgacagatctccttcctgacggctatccagctgactggaatgctatctctaaaacatacgaagcctacaatcaaaactacgagctcgataacctgtggtatctctcgggcctacaacagccggattggcgtgggttagtagctgctgttgacagccattaccaggtctttcacaacggtagttttgactgcccagcaccatgtgaggatgagaatatcaaccatatcttacacgcaaactctgtgtcgggtttacggtggagagttggtggggatcgccatcaagttgccaggaatgagttgtatgttgccacactcccttgcccactttccttggtatgtgacatgaaactaactcctttatagtgcaagcagcatcacccgcgacgtttctcgcattatccgtgataatatcgccacgaagcatggcgttcaaacgtcaaccgacgaccacgctcccatccatccatcaaatttcccgcccctcccaacgggtctaactatgccaaacccgcccacaacctctcaagcgccaatatctttgcgaattaatatcatgcagaacgggaaacgtgtccttccgcgagtagatcttcctgcaggacactgtcccgatcttgagactctgaaacagctactctgccgtcgattcgcgggccagttgccaggtctgccctctgacccttcgctggaccctgcagcctggatgtcttcggttggctggaggtttagagtctggttgcccgagggcctgactcctgtccagaatgacggcgagtggacgatcgcactgctttctgccgggaacgtagactggatggacggtgatctacgagttcttgtagagctggagaacacctcttag

SEQ ID NO: 3 - protein, 657 aa, Aspergillus sojae
MTSSASHHQHPSTSAAEFSAHQTASSSNIDPNGNIATSGYAPNESQLAGLVEAATAAAGQDVSEWAAAAAVAAAAGAAGHQHHLDGYPPDIHIEDDSFADAGFGTGLSAGRQLRAPGPSPNEHSQPSGLSRTVSKKRKRDGPLDPALTASGPGGHQQPHQHNSHHYGGETLDIRSAPPQSLSEARAVGLHSAAALFRQPSSNKKYTRPPMSKLFASLELSPENFLHLQAAAKSYMLDDKHPERRECVGQRGKGDTEMVKLRLWNCVRHFLEIEGHGERFFGENVVNEGMGPRTYVWPRDQQKIIALVIPLLRRMVTNERQRQYAVETRKGGGSEERRRRKTEDSLQNMNSASPPKFPVEEQLQMHAQHHPPEGYAPTHPELGATSQDMELGLTDLLPDGYPADWNAISKTYEAYNQNYELDNLWYLSGLQQPDWRGLVAAVDSHYQVFHNGSFDCPTPCEDENINHILHANSVSGLRWRVGGDRHQVSRNEFASSITRDVSRIIRDNIATKHGVQTSTDDHAPIHPSNFPPLPTGLTMPNPPTTSQAPISLRINIMQNGKRVLPRVDLPAGHCPDLDTLKQLLCRRFAGQLPGLPSDPSLDPAAWMSSVGWRFRVWLPEGLTPVQNDGEWTIALLSAGNVDWMDGDLRVLVELENTS

SEQ ID NO: 4 - DNA, 2038 bp, Aspergillus sojae
  source 1..2038: mol_type = genomic DNA
atgacgtcttctgcttcccatcaccaacatccttcgacttcagccgctgaattttccgctcaccaaaccgcttcttcctccaacatcgacccgaacggtaacattgccacgagtggatatgcgccaaatgaaagccaacttgctgggctggtagaagctgctactgcagcggctggccaggatgtatcggaatgggcggccgccgctgcagtcgctgctgcagctggtgctgccggacatcagcatcatttagacggctaccccccggatattcatatcgaagatgatagttttgcagatgcaggttttgggacagggttgagcgctggaagacagttacgagcacccgggccatcccccaacgaacatagccagccttcgggactgtcaagaactgtgtcaaagaagagaaagagagatggccctctcgacccagccttaacagcgtctggacctggtggtcaccagcagccccatcagcacaattctcatcattatggtggtgagactctagatatccggtctgcgcctccccagtccttatcggaggcgcgcgctgttggtttacattccgcagctgctttgttccgtcaaccctcgagcaacaagaagtacacacgaccacctatgtcgaagctttttgcttcactcgaactatcaccggagaacttcctccacttacaagccgctgctaagtcatatatgctagatgacaagcatccagaacgacgtgagtgtgtcggtcaacgtggcaagggagacacggaaatggttaaattgagactttggaattgtgtgcgccactttctcgaaattgaggggcatggtgaacgatttttcggtgaaaatgtagtcaacgagggcatgggtcccaggacctatgtatggccccgggaccagcaaaaaatcattgcacttgtcattccactgctacggcgtatggtcaccaatgaacgacagagacaatatgcagtggagacgaggaaggggggtggatccgaggagcgacgacgaaggaaaaccgaagacagtctccagaatatgaatagtgctagtcctccgaagttccccgttgaggaacaactccagatgcatgcgcaacatcatcctcccgaggggtatgcgccaacacaccccgagttgggggcaacttcccaagacatggagttgggcttgacagacctccttcctgacggctatccagctgactggaatgctatctctaaaacatacgaagcctacaatcaaaactacgagctcgataacctgtggtatctctcgggcctgcaacagccggattggcgtgggttagtagctgctgttgacagccattaccaagtctttcacaacggtagttttgactgcccaacaccatgtgaggatgagaatatcaaccatatcttacacgcaaactctgtgtcgggtttacggtggagagttggtggggatcgccatcaagtttccaggaatgagttgtatgttgccacactcccttgcccattttcctcggtatgtgacatgaaactaactcctgtatagtgcaagcagtatcacccgcgacgtttctcgcattatccgtgataatatcgccacgaagcatggcgttcaaacgtcaaccgacgaccacgcgcccatccatccatcaaatttcccgcccctcccaacgggtctaactatgccaaacccgcccacaacctctcaagcgccaatatctttgcgaatcaatattatgcagaacgggaaacgtgtccttccgcgagtagatcttcctgcaggacactgtcccgatcttgacactctaaaacagctactctgccgtcgattcgcgggccagttgccaggtctaccctctgacccttcgctggaccctgcagcctggatgtcttcggttggctggagatttagagtctggttgcccgagggcctgactcctgtccagaatgacggcgagtggacgatcgcactcctttctgccgggaacgtagactggatggacggtgatctacgagttcttgtagagctggagaacacctcttag

SEQ ID NO: 5 - protein, 658 aa, Aspergillus tamarii
MTSSASHHQHPSTSAAEFSAHQTAPSSNIDPNGNIATSGYAPNESQLAGLVEAATAAADQDVSEWAAAAAVAAAAGAAGHQHHLDGYPPDIHIEDDSFADAGFGTGLGAGRQLRAPGPSPNEHSQPSGLSRTVSKKRKRDGPLDPALTASGPGGHQQQPHQHTSHHYGGESLDIRSAPPQSLSEARAVGLHSAAALFRQPSSNKKYTRPPMSKLFASLELSPENFLHLQAAAKAYMLDDKHPERRECVGQRGKGDTEMVKLRLWNCVRHFLEIEGHGERFFGENVVNEGMGPRTYVWPRDQQKIIALVIPLLRRMVTNERQRQYAVETRKGGGSEERRRRKTEDSLHNMNSASPPKFPVEEQLQMHAQHHPPEGYAPTHPELGATSQDLELGLTDLLPDGYPADWDAISKTYEAYNQNYELDNLWYISGLQQPDWRGLVAAVDSHYQVFHNGSFDCPTPCEDENINHILHANSVSGLRWRLGGDRNQVARNEFASSITRDLSRIIRDNIATKHGVQTPTDDHASMHPSHFPPLPTGLNMPNPPTTSQAPISLRINIMQNGKRVLPRVDLPAGHCPDLEALKQILCRRFAGQLPGLPSDPSLDPAAWMSSVGWRFKVWLPEGLTPVQNDGEWTIALLSAGNVDWMDGDLRVLVELESTS

SEQ ID NO: 6 - DNA, 2041 bp, Aspergillus tamarii
  source 1..2041: mol_type = genomic DNA
atgacgtcttctgcctcccatcaccaacatccttcgacttcagccgctgagttttctgctcatcaaaccgcaccttcctctaacatcgacccgaacggtaacatcgccacgagtggatatgctccaaatgaaagtcaacttgctgggctggtagaagctgctacggcagcggctgaccaagacgtatcggaatgggcggccgccgctgccgtcgctgccgccgctggtgccgccgggcatcagcatcatctagacggctaccctccggatattcatatcgaagatgatagctttgcagatgcaggttttgggacagggctgggcgctggaagacagttacgggcaccagggccatcccccaacgaacatagtcagccttcgggactatcaagaacggtgtcaaagaagagaaagagagacggccctctcgacccagccttaacagcgtctggacctggtggtcaccagcagcaaccccaccagcacacttcgcatcattatggtggcgaaagtctcgatatccggtctgcacctccccagtccttatcggaagcgcgtgctgttggtttacattccgcagctgctttgttccgtcaaccctcgagcaacaagaagtatacccgaccacctatgtcgaagctttttgcttcattagaactatcaccagagaacttcctacatttacaagccgctgctaaggcatatatgctcgatgacaagcatccagaacgacgtgagtgtgtcggtcagcgtggcaagggagacacggaaatggttaaattgaggctttggaattgtgtgcgccacttcctcgaaattgagggccatggtgaacgttttttcggtgaaaatgtagtcaacgagggcatgggtcccaggacctatgtatggccccgggaccagcaaaaaatcattgcgctggtcattccacttctacggcgtatggtcaccaatgaacgacagaggcaatatgcagttgagacgaggaaggggggtggatcagaggagcgacgacgaaggaaaacagaagatagtctccacaatatgaatagtgccagtccccccaagttccccgttgaggaacaactccagatgcacgcgcaacaccatcctcccgagggctatgcgccaacgcaccccgagttgggggcgacttcccaagacctggagttgggcctcacagatctgcttcctgatggctacccagctgactgggatgccatctctaaaacatacgaagcctacaatcagaactacgagctcgacaacctgtggtatatctcgggcctacaacagccagattggcgtgggttagtagcggctgttgacagccattatcaggtctttcacaacggtagttttgactgccccacaccatgtgaggatgagaatatcaaccatattttacatgcaaactctgtgtcgggtttacggtggaggcttggtggagatcgcaatcaagttgccaggaatgagttgtatgttgccacactcccatgaccactttgctcggtatgtgacatgaaactaactcccttacagtgcaagcagtatcacccgcgacctttctcgcattatccgtgataatatcgccacgaagcatggcgttcaaacgcctaccgacgaccacgcgtccatgcatccatcacatttcccgcccctcccaacgggtctaaatatgccaaatccgccaacaacctctcaagcgccaatatctttgcgaatcaatatcatgcagaacggcaaacgtgtccttccgcgggtagatcttcctgcaggacactgtcccgatcttgaggctttgaaacagatactgtgccgtcgattcgcgggccagttgccaggtctaccgtctgacccttcattggaccctgcagcctggatgtcttcggttggctggagattcaaagtctggttgcccgagggcctgactcctgtccaaaatgacggcgagtggacgatcgcactcctctctgccgggaacgtagactggatggacggtgatctacgagttcttgtagagctggagagcacctcttag

SEQ ID NO: 7 - protein, 680 aa, Aspergillus luchuensis
MASTSNSNHQHPPSTSAAEFSTNPTTSANVDPNTHLANSGYAPSENQLAGLVEAATAAAGQEVSDWAAAAAVAAAAGAAGLQHHLEYGPDTHIDEDSFADASFGAGMGTQRQMRGPGSTSMSEHGQPSGGLTRVPTKKRKRNEDALDPALTAGAAVGLAGTHHPHHQQQQQQHHQHAHHYGGEGLGVAPSQSLSEARAVGLHSAAALFRQPSSNKKYTRPPMSKLFASLELSPENFLHLQAAAKAYMLDDRHPERRDCVGQRGKGDTEMVKLRLWNCVRHFLEVEGHGERFFGENVVNEGMGPRTYIWPRDQQKIISLVIPLLRRMVTNERQRQYAVETRKGGGTEERRRRKTEDSLQNLNATTPTDDQLHMHSHHHLPDDYTSAQTGLGAPQPQLGTGSQLDLGLTDLLLDGYSADWDSFSKSYDLYNHNYELDNLWYISGLQQPDWRGLVAAIDSHFQVIHNGGYDCPSPCEDQNLHRILNADATSDLRWRVGGNSDRPARNEFASSITRDISRIIRDSLATQHNVHQSPHSQAPVPQPQPFPPPNFPPLPSAVSGNTGSSPSPPTNVSLRINILQDGKRTHPRFDIPGNQCTDLETLKQLISRKFAGQLPGLPSEVNMDWVSQLPWKFKVWLPDGLAPVQNDNEWAMALVSASNVDWMDGDLRVLVELDGTASAPSS

SEQ ID NO: 8 - DNA, 2098 bp, Aspergillus luchuensis
  source 1..2098: mol_type = genomic DNA
atggcatcgacttctaattcaaaccatcaacaccctccgtcgacttcggctgccgagttctcgaccaacccgaccacctccgccaatgtcgaccctaacacccacctcgcaaacagcggatatgcgcccagtgagaatcagctagctggcttagtggaggcagccacagctgctgccggtcaggaggtctccgattgggctgctgccgccgctgttgctgcggcggcgggcgccgcgggcctccagcatcacctcgagtatggtccggatacccacatcgatgaggatagttttgcagatgcaagttttggtgctggaatggggacgcagcggcagatgcgcggacctgggtctacctctatgagtgaacatggccagccctccggtgggttgaccagggtgccaacgaagaaacggaagaggaatgaggatgcgctggatccggccttgactgcgggagctgccgtcggcctcgctggcacgcatcatcctcaccaccaacagcagcagcagcaacatcaccagcatgcgcatcactacggtggggagggtctgggcgtcgcgccgtcgcagtctctctccgaagctcgcgctgtgggtctgcattccgccgcagccttgttccgccaaccgtcgagtaacaagaagtacacccgtccgccgatgtcgaagttatttgcgtcgctggaactttcgccggaaaacttcttgcatctgcaggcggcggctaaggcatatatgctggatgatcgccatccggaacggcgcgattgtgttggtcagcgtggaaagggtgataccgagatggttaagttgcggttgtggaactgcgtgcgtcactttcttgaggtcgaaggccatggtgagcgcttcttcggagagaatgtggtcaacgagggcatggggcctaggacatacatctggccccgggaccagcagaagatcatctctttggttattcctttgctgcgccgaatggtcacaaacgagcgccagcggcagtatgcagtggagactagaaaaggtggcggcacagaagagcgacggagacgcaagacagaggacagtctgcaaaacctgaacgcgaccaccccgacagatgatcaactccacatgcattcacaccaccatcttccggacgattatacttctgcacagaccgggctgggggcaccacaaccgcagctcggtaccgggtctcagttggatctgggtctgactgatctcctgctggatggttactcggctgactgggattcgttctcgaagtcgtatgacctgtacaatcataattatgaacttgacaacctttggtacatctcaggtctccaacagccggattggcgtggactggtcgctgccattgatagccacttccaggtcattcacaacggcggctacgactgtccgtcaccatgtgaggatcagaatttgcatcgcattttgaatgcagatgccacgtcggacttgcgttggcgtgttggcgggaattcagaccgtcctgccagaaatgaattgtatgttcccaacataacagtcaacaatttgtgtatatcactaacaacccgatagtgccagcagcatcacccgtgacatctcccgaatcatccgagacagcctagcgacccagcacaatgtccatcaatccccccacagccaggcaccagtgccccagcctcagcccttccctcctcccaatttcccgcctctccccagcgctgtctccggaaacaccggctcttctccgtctcctccaaccaacgtttcactccgaatcaacatcctacaggacggaaaacgcacgcatccccgtttcgacattcccggaaaccaatgcaccgatcttgaaaccctcaagcaactcatctcccgcaaatttgccggccaactgccaggtctcccatccgaagtaaacatggactgggtctctcaacttccctggaaattcaaggtctggctaccagatggactggccccggtgcaaaatgacaacgagtgggcaatggccctagtctcagctagcaatgtagactggatggatggtgatctccgagttctggttgaattagacgggacagcatcggcgccgtcgtcttga

SEQ ID NO: 9 - protein, 680 aa, Aspergillus niger
MASTSNSNHQHPPSTSAAEFSTNPTTSANVDPNTHLANSGYAPSENQLAGLVEAATAAAGQEVSDWAAAAAVAAAAGAAGLQHHLEYGPDTHIDEDSFADASFGAGMGTQRQMRGPGSTSMSEHGQPSGGLTRVPTKKRKRNEDALDPALTAGAAVGLAGTHHPHHQQQQQQHHQHAHHYGGEGLGVAPSQSLSEARAVGLHSAAALFRQPSSNKKYTRPPMSKLFASLELSPENFLHLQAAAKAYMLDDRHPERRDCVGQRGKGDTEMVKLRLWNCVRHFLEVEGHGERFFGENVVNEGMGPRTYIWPRDQQKIISLVIPLLRRMVTNERQRQYAVETRKGGGTEERRRRKTEDSLQNLNATTPTDDQLHMHSHHHLPDDYTSAQTGLGAPQPQLGTGSQLDLGLTDLLLDGYSADWDSFSKSYDLYNHNYELDNLWYISGLQQPDWRGLVAAIDSHFQVIHNGGYDCPSPCEDQNLHRILNADATSDLRWRVGGNSDRPARNEFASSITRDISRIIRDSLATQHSVHQSPHSQAPVPQPQPFPPPNFPPLPSAVSGNTGSSPSPPTNVSLRINILQDGKRTHPRFDIPGNQCTDLETLKQLISRKFAGQLPGLPSEVNMDWVSQLPWKFKVWLPDGLAPVQNDNEWAMALVSASNVDWMDGDLRVLVELDGTASAPSS

SEQ ID NO: 10 - DNA, 2098 bp, Aspergillus niger
  source 1..2098: mol_type = genomic DNA
atggcatcgacttctaattcaaaccatcaacaccctccgtccacttcggctgccgagttctcgaccaacccgaccacctccgccaatgtcgaccctaacacccacctcgcaaacagcggatatgcgcccagtgagaatcagctagctggcttagtggaggcagccacagctgctgccggtcaagaggtctctgactgggctgctgctgccgctgtcgctgcggcggcgggggctgcgggcctccagcatcacctcgagtatggtccggatacccacatcgatgaggatagttttgcagatgcaagttttggtgctggaatggggacgcagcggcagatgcgcggacctgggtctacctctatgagtgaacatggccagccctccggtgggttgaccagggtgccaacgaagaaacggaagaggaatgaggatgcgctggatccggccttgactgcgggagctgccgtcggcctcgctggcacgcatcatcctcaccaccaacagcagcagcagcaacatcaccagcatgcgcatcactatggtggggaggggctcggcgtcgcgccgtcgcagtctctctccgaagctcgcgctgtgggtctgcattccgccgcagccttgttccgccaaccgtcgagtaacaagaagtacacccgtccgccgatgtcgaagttatttgcgtcgctggaactttcgccggaaaacttcttgcatctgcaggcggcggctaaggcatatatgctcgatgatcgccatccggaacggcgcgattgtgtcggtcagcgtggaaagggtgataccgagatggttaagttgcggttgtggaactgcgtgcgtcactttcttgaggtcgaaggccatggtgagcgcttcttcggagagaacgtggtcaacgagggcatggggcctaggacatacatctggccccgggaccagcagaagatcatctctttggttattcctttgctgcgccgaatggtcacaaacgagcgccagcggcagtatgcagtggagactagaaaaggtggcggcacagaagagcgacggagacgcaagacagaggacagtctgcaaaacctgaacgcgaccaccccgacagatgatcaactccacatgcattcacaccaccatcttccggacgattatacttccgcacagaccgggctgggggcaccacaaccgcagctcggcaccgggtctcagttggatctgggtctgactgatctcctgctggatggttactcggctgactgggattcgttctcgaagtcgtatgacctgtacaatcataattatgaacttgacaacctgtggtacatctcgggtctccaacagccggattggcgtggactggtcgctgccattgatagccacttccaggtcattcacaacggcggctacgactgtccgtcaccatgtgaggatcagaatttgcatcgcattttgaatgcagatgccacgtcggacctgcgttggcgtgttggcgggaattcagaccgtcctgccagaaatgaattgtatgttcccaacataacagtcaacaatttgtgtatatcactaacaacccgatagtgccagcagcatcacccgtgacatctcccgaatcatccgagacagcctagcgacacagcacagtgtccatcaatccccccacagccaggcaccagtgccccagcctcagcccttccctcctcccaatttcccgcctctccccagcgctgtctccggaaacaccggctcttctccgtctcctccaaccaacgtttcactccgaatcaacatcctacaggacggaaaacgcacgcatccccgtttcgacattcccggaaaccaatgcaccgatcttgaaaccctcaagcaactcatctcccgcaaatttgccggccaactgccaggtctcccatccgaagtaaacatggactgggtctctcaacttccctggaaattcaaggtctggctaccagatggactggccccggtgcaaaatgacaacgaatgggcaatggccctagtctcagctagtaatgtagactggatggatggtgatctccgagttctggttgaattggacgggacagcatcggcgccgtcgtcttga

SEQ ID NO: 11 - protein, 679 aa, Aspergillus nidulans
MTSTAPTNQQHPPSGPSSEFSGNQPPASSGADQSTHISTSGYAPSENQLAGLVEAATAAAGQDVSEWAAAAAVAAAAGAAGNQHHLDGYAPDIQLDEDGFDEGGYAGMTGARHYRGPGSTSGNEHGQSSGLARSGTKKRKRNEDALDPALAAASASLGQHHGQPQHQNQSQHHVHHASPYPGEGLEIRNTPPQTLADARAVGLHSAAALFRQTSTNKKYTRPPMSKMFTSLELSPENFLHLQAAAKAYMLDDRHPERRDCVGQRGKGDTEMVKLRLWNCVRHFLEVEGNGPRFFGEHVVNEGMPPRTYVWPRDQQKIISLVIPLLRRMVTNERQRQYAVETRKGGVEARRRRKTEDSIQDFRSASPPKFSSEDHLQMQADHQLPDGYSSTQHPLSASAPPPPHSEPSVQVTELGLTDLILDGYSTDLDSISKSYDSYNHNYELDNLWSLSGLHLGDWRGLVAAVDSHYQILHEGDYNCSGCCEDGNIGRILNSTSTADLRWRIGGDPARNEFASSITRDVSRVIRDNLAARQGAQNHTSLPQTQPIPPPLPFSHSSDLSNPNPPPAQSPLRLRINILQNGKRILPSYDLPATQGPDVTTVRQLVARKFAGELPGIPSDLNSDSNTWNASISWKFKVWLPEGLVLIENDGDWTLALLAAEKVDWLDGELKVLVEIEDENQ

SEQ ID NO: 12 - DNA, 2100 bp, Aspergillus nidulans
  source 1..2100: mol_type = genomic DNA
atgacgtctaccgctccgacaaaccaacaacatcccccatccggaccatcaagcgaattctctggtaatcaaccacccgcttcatccggcgcagaccagagtacacacatttcaacgagtggatatgcgccgagcgagaatcagcttgctggcttggtagaggccgctacagctgcggccggccaagacgtgtcggagtgggcagcggcagcagcagtcgccgcagcagctggcgccgcagggaatcaacatcatctggacgggtacgcgcctgacattcaattggacgaggatggctttgacgagggaggctatgcgggcatgactggcgcccgacattatcgtggacctggttcaacgtctggcaatgagcacggtcaatcctcgggtttggctcgatcggggacgaagaagagaaagagaaacgaggatgctcttgatccggctttggctgccgcaagcgcgagtctcggccagcatcacggtcaaccgcaacatcagaatcaaagtcaacaccacgtccaccatgcaagcccgtacccaggggagggactggaaattcgcaatactccgccgcaaacgcttgcggatgcccgcgccgttggactgcactccgctgcagcactattccgtcaaacctcaaccaacaagaagtatactaggcctcccatgtcgaagatgttcacttctctggagctatcgccggaaaattttctacatttacaagctgcggctaaagcatacatgctagatgataggcatccggagcgccgtgactgcgtaggccagcgcgggaaaggagatacagagatggtcaaattacggttatggaactgtgtccgtcacttcctcgaggtcgagggcaatggcccgcgattcttcggtgaacatgtggtcaacgagggtatgcctcctcggacatacgtctggccaagggaccaacagaaaatcatctcactcgttattccgttgttgaggcgcatggtcacaaacgaacgacaacgacaatacgctgtcgaaaccaggaaaggtggcgtggaggcacgaagaaggcgaaaaacagaagatagtatccaagacttccgcagtgcgagtccacccaagttctcatccgaggaccaccttcagatgcaggcggatcatcagcttcccgatggatatagctcaactcaacaccctctatcagcgtctgccccgccaccacctcacagtgaaccatctgtgcaggtcacagaactgggccttactgatcttatcctggatggttatagtacagacttggattctatttcaaagtcgtatgattcgtacaaccataactatgaacttgataacctatggtctctctcgggcctacatttaggcgattggcgcggtcttgtggctgcagttgatagccactatcagattcttcacgagggagactataattgcagcggttgttgtgaagacggcaacataggacgcattctcaattcgactagcaccgcagatctacgatggcgtattggcggcgaccctgccaggaatgagttgtaagtctgcgacatatcatctgcatgcgaagaaaaccactaaacttttccctcctgcagcgcaagtagcatcacccgcgacgtctcacgggttatccgcgacaatctagcagctaggcaaggcgctcaaaaccacacatcactgccccaaacccagcctatcccaccgccccttcccttttctcattcatccgacctttcaaaccccaatccccctcccgcccaatcgcctctccgcctccgcatcaacattctgcaaaacgggaagcgcatcctcccttcctatgaccttcccgctactcagggtccagacgtcacaaccgtgcgccagctcgtagcgcgcaaattcgccggtgaacttcctggtatcccttcagacctgaattcggactccaacacctggaacgcatccataagctggaaatttaaagtttggctaccggaggggcttgttctcattgagaatgatggcgattggacgctggcgctccttgccgcggagaaggtggactggcttgatggcgagctgaaggttcttgttgaaattgaggatgagaatcagtag

SEQ ID NO: 13 - protein, 69 aa, Synthetic Construct
YEAYNQNYELDNLWYLSGLQQPDWRGLVAAVDSHYQVFHNGSFDCPAPCEDENINHILHANSVSGLRWR

SEQ ID NO: 14 - protein, 57 aa, Synthetic Construct
YEAYNQNYELDNLWYLSGLQQPDWRGLVAAVDSHYQVFHNGSFDCPAPCEDENINHI

SEQ ID NO: 15 - protein, 52 aa, Synthetic Construct
YEAYNQNYELDNLWYLSGLQQPDWRGLVAAVDSHYQVFHNGSFDCPAPCEDE

SEQ ID NO: 16 - protein, 34 aa, Synthetic Construct
YEAYNQNYELDNLWYLSGLQQPDWRGLVAAVDSH

SEQ ID NO: 17 - protein, 18 aa, Synthetic Construct
SGLQQPDWRGLVAAVDSH

SEQ ID NO: 18 - protein, 8 aa, Synthetic Construct
DWRGLVAA

SEQ ID NO: 19 - protein, 18 aa, Synthetic Construct
SGLXXXDWRGLVAAXDSH

SEQ ID NO: 20 - protein, 14 aa, Synthetic Construct
SGLQQPDWRGLVAA

SEQ ID NO: 21 - protein, 26 aa, Synthetic Construct
ELDNLWYLSGLQQPDWRGLVAAVDSH

SEQ ID NO: 22 - DNA, 45 bp, Synthetic Construct
  source 1..45: mol_type = other DNA
cggtacccggggatcttagatcaagtgaggaacacctcctaggca

SEQ ID NO: 23 - DNA, 45 bp, Synthetic Construct
  source 1..45: mol_type = other DNA
tagcaataagcccaacggccagagatatagtcactcaattccgtt

SEQ ID NO: 24 - DNA, 40 bp, Synthetic Construct
  source 1..40: mol_type = other DNA
tcttctgaggtgcagatctcagtgcccgatccgggtagag

SEQ ID NO: 25 - DNA, 40 bp, Synthetic Construct
  source 1..40: mol_type = other DNA
cgactctagaggatctccgagagcaacagcgacactctca

SEQ ID NO: 26 - DNA, 28 bp, Synthetic Construct
  source 1..28: mol_type = other DNA
ttgggcttattgctatgtccctgaaagg

SEQ ID NO: 27 - DNA, 32 bp, Synthetic Construct
  source 1..32: mol_type = other DNA
ctgcacctcagaagaaaaggatgatcaatacc

SEQ ID NO: 28 - DNA, 24 bp, Synthetic Construct
  source 1..24: mol_type = other DNA
caacagccggattggcgtgggtta

SEQ ID NO: 29 - DNA, 30 bp, Synthetic Construct
  source 1..30: mol_type = other DNA
gagataccacaggttatcgagctcgtagtt

SEQ ID NO: 30 - DNA, 30 bp, Synthetic Construct
  source 1..30: mol_type = other DNA
taccaggtctttcacaacggtagttttgac

SEQ ID NO: 31 - DNA, 30 bp, Synthetic Construct
  source 1..30: mol_type = other DNA
gtagttttgattgtaggcttcgtatgtttt

SEQ ID NO: 32 - DNA, 22 bp, Synthetic Construct
  source 1..22: mol_type = other DNA
tcggcctcgccttcttcatcgt

SEQ ID NO: 33 - DNA, 31 bp, Synthetic Construct
  source 1..31: mol_type = other DNA
taagtcatgtccgtaatgggcatcaaaaggg

SEQ ID NO: 34 - DNA, 36 bp, Synthetic Construct
  source 1..36: mol_type = other DNA
cggtacccggggatccaccgcagccaatccccagtt

SEQ ID NO: 35 - DNA, 39 bp, Synthetic Construct
  source 1..39: mol_type = other DNA
tagcaataagcccaagacatcgggaattgggtcatccgg

SEQ ID NO: 36 - DNA, 42 bp, Synthetic Construct
  source 1..42: mol_type = other DNA
cgactctagaggatcgaccaccttggaagaaagctgacctga

SEQ ID NO: 37 - DNA, 22 bp, Synthetic Construct
  source 1..22: mol_type = other DNA
ctgcaacagccggattggcgtg

SEQ ID NO: 38 - DNA, 28 bp, Synthetic Construct
  source 1..28: mol_type = other DNA
cgagagataccacaggttatcgagctcg

SEQ ID NO: 39 - DNA, 30 bp, Synthetic Construct
  source 1..30: mol_type = other DNA
gttgacagccattaccaagtctttcacaac

SEQ ID NO: 40 - DNA, 30 bp, Synthetic Construct
  source 1..30: mol_type = other DNA
taccaagtctttcacaacggtagttttgac

SEQ ID NO: 41 - DNA, 22 bp, Synthetic Construct
  source 1..22: mol_type = other DNA
gccgtgggcataggcacgattg

SEQ ID NO: 42 - DNA, 27 bp, Synthetic Construct
  source 1..27: mol_type = other DNA
gctagcatcacatctcacgacacgtcc

SEQ ID NO: 43 - protein, 18 aa, Synthetic Construct
SGLXXXXWXGXXAAXDSH

SEQ ID NO: 44 - protein, 34 aa, Synthetic Construct
YXAYNXXXELDXLXXXSGLXXXDWRGLVAAXDSH

SEQ ID NO: 45 - protein, 57 aa, Synthetic Construct
YXAYNXXXELDXLXXXSGLXXXDWRGLVAAXDSHXXXXHXGXXXCXAPCEXENXXXI

SEQ ID NO: 46 - DNA, 45 bp, Synthetic Construct; identical to SEQ ID NO: 22
  source 1..45: mol_type = other DNA

SEQ ID NO: 47 - DNA, 28 bp, Synthetic Construct
  source 1..28: mol_type = other DNA
gctgttgtaggctcgagagataccacag

SEQ ID NO: 48 - DNA, 28 bp, Synthetic Construct
  source 1..28: mol_type = other DNA
ctgtggtatctctcgagcctacaacagc

SEQ ID NO: 49 - DNA, 28 bp, Synthetic Construct
  source 1..28: mol_type = other DNA
attctcatcctcaaatggtgctgggcag

SEQ ID NO: 50 - DNA, 29 bp, Synthetic Construct
  source 1..29: mol_type = other DNA
gactgcccagcaccatttgaggatgagaa

SEQ ID NO: 51 - DNA, 36 bp, Synthetic Construct
  source 1..36: mol_type = other DNA
tttcttctgaggtgcctcgcacagccatgctgtgcc

SEQ ID NO: 52 - DNA, 24 bp, Synthetic Construct
  source 1..24: mol_type = other DNA
gctgttgcaggctcgagagatacc

SEQ ID NO: 53 - DNA, 24 bp, Synthetic Construct
  source 1..24: mol_type = other DNA
ggtatctctcgagcctgcaacagc

SEQ ID NO: 54 - DNA, 28 bp, Synthetic Construct
  source 1..28: mol_type = other DNA
ttgggcttattgctatgtccctgaaagg

SEQ ID NO: 55 - DNA, 30 bp, Synthetic Construct
  source 1..30: mol_type = other DNA
gcacctcagaagaaaaggatgatcaatacc

SEQ ID NO: 56 - DNA, 45 bp, Synthetic Construct
  source 1..45: mol_type = other DNA
cggtacccggggatccccgactgtgcaatatctccaattcctatc

SEQ ID NO: 57 - DNA, 45 bp, Synthetic Construct
  source 1..45: mol_type = other DNA
tagcaataagcccaaaggatggctacgatatcatatgcagtgtct

SEQ ID NO: 58 - DNA, 44 bp, Synthetic Construct
  source 1..44: mol_type = other DNA
tcttctgaggtgcggagtctgaactcgaggagcagttcaaggga

SEQ ID NO: 59 - DNA, 30 bp, Synthetic Construct
  source 1..30: mol_type = other DNA
ggctgttggagactcgagatgtaccacagg

SEQ ID NO: 60 - DNA, 28 bp, Synthetic Construct
  source 1..28: mol_type = other DNA
tgtggtacatctcgagtctccaacagcc

SEQ ID NO: 61 - DNA, 44 bp, Synthetic Construct
  source 1..44: mol_type = other DNA
cgactctagaggatcaagtcgcccatgtaacgaatcaacgctaa

SEQ ID NO: 62 - DNA, 23 bp, Synthetic Construct
  source 1..23: mol_type = other DNA
cgtcagtccgcttcaatgttacc

SEQ ID NO: 63 - DNA, 30 bp, Synthetic Construct
  source 1..30: mol_type = other DNA
gttcgatgtgtatactagggttcagagtag

SEQ ID NO: 64 - DNA, 25 bp, Synthetic Construct
  source 1..25: mol_type = other DNA
ttgggcttattgctatgtccctgaa

SEQ ID NO: 65 - DNA, 24 bp, Synthetic Construct
  source 1..24: mol_type = other DNA
ccgcacctcagaagaaaaggatga

SEQ ID NO: 66 - DNA, 42 bp, Synthetic Construct
  source 1..42: mol_type = other DNA
cggtacccggggatcccaagccctctgggttaacatacacga

SEQ ID NO: 67 - DNA, 45 bp, Synthetic Construct; identical to SEQ ID NO: 57
  source 1..45: mol_type = other DNA

SEQ ID NO: 68 - DNA, 42 bp, Synthetic Construct
  source 1..42: mol_type = other DNA
tcttctgaggtgcagcgaagaagtctgaactcgaggagcagt

SEQ ID NO: 69 - DNA, 41 bp, Synthetic Construct
  source 1..41: mol_type = other DNA
cgactctagaggatctcgcccatgtaacgaatcaacgctaa

SEQ ID NO: 70 - DNA, 22 bp, Synthetic Construct
  source 1..22: mol_type = other DNA
caacagccggattggcgtggac

SEQ ID NO: 71 - DNA, 30 bp, Synthetic Construct
  source 1..30: mol_type = other DNA
gatgtaccacaggttgtcaagttcataatt

SEQ ID NO: 72 - DNA, 23 bp, Synthetic Construct
  source 1..23: mol_type = other DNA
ttccaggtcattcacaacggcgg

SEQ ID NO: 73 - DNA, 30 bp, Synthetic Construct
  source 1..30: mol_type = other DNA
ataattatgattgtacaggtcatacgactt

SEQ ID NO: 74 - DNA, 27 bp, Synthetic Construct
  source 1..27: mol_type = other DNA
agaataagggtcacgaggtgatggtct

SEQ ID NO: 75 - DNA, 30 bp, Synthetic Construct
  source 1..30: mol_type = other DNA
tgcatcatgaggtagaactttaggtgctac

SEQ ID NO: 76 - DNA, 25 bp, Synthetic Construct
  source 1..25: mol_type = other DNA
ttacggtggagagttggtggggatc

SEQ ID NO: 77 - DNA, 25 bp, Synthetic Construct
  source 1..25: mol_type = other DNA
ttgtaggcccgagagataccacagg

SEQ ID NO: 78 - DNA, 21 bp, Synthetic Construct
  source 1..21: mol_type = other DNA
acgtcaaccgacgaccacgct

SEQ ID NO: 79 - DNA, 25 bp, Synthetic Construct
  source 1..25: mol_type = other DNA
gtcagctggatagccgtcaggaagg